European Patent Specification EP 3 773 460 B1, published December 6, 2023. Title: USE OF A PEPTIDE FOR THE TREATMENT OF EPIDERM. Applicant: SEDERMA. The sequence listing filed with the application follows.

SEQUENCE LISTING (24 sequences)

SEQ ID NO: 1 - protein, 5 aa, artificial sequence
  synthetic peptide
  MOD_RES (1)..(1): amidation by a Palmitoyl chain on the N terminal end
KTTKS

SEQ ID NO: 2 - protein, 4 aa, artificial sequence
  synthetic peptide
  MOD_RES (1)..(1): amidation by a Palmitoyl chain on the N terminal end
GQPR

SEQ ID NO: 3 - protein, 6 aa, artificial sequence
  synthetic peptide
  MOD_RES (1)..(1): amidation by a Palmitoyl chain on the N terminal end
VGVAPG

SEQ ID NO: 4 - protein, 4 aa, artificial sequence
  synthetic peptide
  MISC_FEATURE (1)..(1): Xaa being a lysine, ornithine, diaminobutyric acid, diaminopropionic acid or an hydroxylated derivative thereof
  MOD_RES (1)..(1): X = -CO-R1 or -SO2-R1 or biot group, R1 = C1-C24 group
  MOD_RES (4)..(4): Z = -OR1, -NH2, -NHR1 ou -NR1R2 ; R1, R2 = C1-C24 group
  MISC_FEATURE (4)..(4): Xaa being a lysine, ornithine, diaminobutyric acid, diaminopropionic acid or an hydroxylated derivative thereof
XTFX

SEQ ID NO: 5 - protein, 4 aa, Artificial sequence
  Synthetic peptide
  MOD_RES (1)..(1): amidation by a Palmitoyl chain on the N terminal end
KTFK

SEQ ID NO: 6 - protein, 4 aa, artificial sequence
  synthetic peptide
RSRK

SEQ ID NO: 7 - protein, 4 aa, artificial sequence
  synthetic peptide
GQPR

SEQ ID NO: 8 - protein, 4 aa, Artificial sequence
  Synthetic peptide
KTAK

SEQ ID NO: 9 - protein, 4 aa, Artificial sequence
  Synthetic peptide
KAYK

SEQ ID NO: 10 - protein, 4 aa, Artificial sequence
  Synthetic peptide
KFYK

SEQ ID NO: 11 - protein, 5 aa, artificial sequence
  synthetic peptide
KTTKS

SEQ ID NO: 12 - protein, 6 aa, artificial sequence
  Synthetic peptide
GKTTKS

SEQ ID NO: 13 - protein, 6 aa, artificial sequence
  synthetic peptide
VGVAPG

SEQ ID NO: 14 - protein, 4 aa, Artificial sequence
  Synthetic peptide
  MOD_RES (1)..(1): amidation by a Elaidoyl chain on the N terminal end
KTAK

SEQ ID NO: 15 - protein, 4 aa, Artificial sequence
  Synthetic peptide
  MOD_RES (1)..(1): amidation by a Elaidoyl chain on the N terminal end
KAYK

SEQ ID NO: 16 - protein, 4 aa, Artificial sequence
  Synthetic peptide
  MOD_RES (1)..(1): amidation by a Elaidoyl chain on the N terminal end
KFYK

SEQ ID NO: 17 - protein, 5 aa, artificial sequence
  synthetic peptide
  MOD_RES (1)..(1): amidation by a Palmitoyl chain on the N terminal end
  MISC_FEATURE (5)..(5): Xaa being either a Proline P or a Leucine L.
YGGFX

SEQ ID NO: 18 - protein, 6 aa, artificial sequence
  synthetic peptide
  MOD_RES (1)..(1): amidation by a Palmitoyl chain on the N terminal end
GKTTKS

SEQ ID NO: 19 - protein, 6 aa, Artificial sequence
  Synthetic peptide
  MOD_RES (1)..(1): amidation by a Palmitoyl chain on the N terminal end
  MISC_FEATURE (6)..(6): Xaa being Trp, Phe, Tyr, Tic, 7-hydroxy-Tic or Tpi
HLDIIX

SEQ ID NO: 20 - protein, 6 aa, artificial sequence
  synthetic peptide
  MOD_RES (1)..(1): Acetylation on the N-terminal end
EEMQRR

SEQ ID NO: 21 - protein, 5 aa, artificial sequence
  synthetic peptide
YAGFL

SEQ ID NO: 22 - protein, 4 aa, artificial sequence
  synthetic peptide
AHSH

SEQ ID NO: 23 - protein, 6 aa, artificial sequence
  synthetic peptide
SIKVAV

SEQ ID NO: 24 - protein, 6 aa, artificial sequence
  synthetic peptide
GPQGPQ